European Patent Specification EP 3 519 595 B1, published August 13, 2025. Title: Means and methods for plant yield enhancement. Applicant: Aphea.Bio NV FUNDACIÓN CENTRO DE EXCELENCIA EN INVESTIGACIÓN DE MEDICAMENTOS INNOVADORES EN ANDALUCÍA, MEDINA. The sequence listing filed with the application follows.

SEQUENCE LISTING (3 sequences)

SEQ ID NO: 1 - DNA, 1384 bp, Streptomyces niveus
agtcgaacgatgaagccttcgggtggattagtggcgaacgggtgagtaacactgtgggcaatctgccctgcactctgggacaagccctggaaacggggtctaataccggataatactgtgcccctcctgggggacggttgaaagctccggcggtgcaggatgagcccgcggcctatcagcttgttggtggggtaatggcctaccaaggcgacgacgggtagccggcctgagagggcgaccggccacactgggactgagacacggcccagactcctacgggaggcagcagtggggaatattgcacaatgggcgaaagcctgatgcagcgacgccgcgtgagggatgacggccttcgggttgtaaacctctttcagcagggaagaagcgaaagtgacggtacctgcagaagaagcgccggctaactacgtgccagcagccgcggtaatacgtagggcgcaagcgttgtccggaattattgggcgtaaagagctcgtaggcggtttgtcacgtcgggtgtgaaagcccggggcttaaccccgggtctgcattcgatacgggcagactagagtgtggtaggggagatcggaattcctggtgtagcggtgaaatgcgcagatatcaggaggaacaccggtggcgaaggcggatctctgggccattactgacgctgaggagcgaaagcgtggggagcgaacaggattagataccctggtagtccacgccgtaaacgttgggaactaggtgttggcgacattccacgtcgtcggtgccgcagctaacgcattaagttccccgcctggggagtacggccgcaaggctaaaactcaaaggaattgacgggggcccgcacaagcagcggagcatgtggcttaattcgacgcaacgcgaagaaccttaccaaggcttgacatacaccggaaagcatcagagatggtgccccccttgtggtcggtgtacaggtggtgcatggctgtcgtcagctcgtgtcgtgagatgttgggttaagtcccgcaacgagcgcaacccttgttctgtgttgccagcatgcctttcggggtgatggggactcacaggagaccgccggggtcaactcggaggaaggtggggacgacgtcaagtcatcatgccccttatgtcttgggctgcacacgtgctacaatggccggtacaatgagctgcgataccgcaaggtggagcgaatctcaaaaagccggtctcagttcggattggggtctgcaactcgaccccatgaagtcggagttgctagtaatcgcagatcagcattgctgcggtgaatacgttcccgggccttgtacacaccgcccgtctagtggcgaaagtcggtaacacccgaagccggtggcccaaccccttggggagggag

SEQ ID NO: 2 - DNA, 1388 bp, Arthrobacter oxydans
tgcaagtcgaacgatgatccggtgcttgcaccggggattagtggcgaacgggtgagtaacacgtgagtaacctgcccttaactctgggataagcctgggaaactgggtctaataccggatatgactgatcatcgcatggtggttggtggaaagctttttgtggttttggatggactcgcggcctatcagcttgttggtgaggtaatggcttaccaaggcgacgacgggtagccggcctgagagggtgaccggccacactgggactgagacacggcccagactcctacgggaggcagcagtggggaatattgcacaatgggcgcaagcctgatgcagcgacgccgcgtgagggatgacggccttcgggttgtaaacctctttcagtagggaagaagcgaaagtgacggtacctgcagaagaagcgccggctaactacgtgccagcagccgcggtaatacgtagggcgcaagcgttatccggaattattgggcgtaaagagctcgtaggcggtttgtcgcgtctgccgtgaaagtccggggctcaactccggatctgcggtgggtacgggcagactagagtgatgtaggggagactggaattcctggtgtagcggtgaaatgcgcagatatcaggaggaacaccgatggcgaaggcaggtctctgggcattaactgacgctgaggagcgaaagcatggggagcgaacaggattagataccctggtagtccatgccgtaaacgttgggcactaggtgtgggggacattccacgttttccgcgccgtagctaacgcattaagtgccccgcctggggagtacggccgcaaggctaaaactcaaaggaattgacgggggcccgcacaagcggcggagcatgcggattaattcgatgcaacgcgaagaaccttaccaaggcttgacatgaaccggaaagacctggaaacaggtgccccgcttgcggtcggtttacaggtggtgcatggttgtcgtcagctcgtgtcgtgagatgttgggttaagtcccgcaacgagcgcaaccctcgttctatgttgccagcacgtgatggtggggactcataggagactgccggggtcaactcggaggaaggtggggacgacgtcaaatcatcatgccccttatgtcttgggcttcacgcatgctacaatggccggtacaaagggttgcgatactgtgaggtggagctaatcccaaaaagccggtctcagttcggattggggtctgcaactcgaccccatgaagtcggagtcgctagtaatcgcagatcagcaacgctgcggtgaatacgttcccgggccttgtacacaccgcccgtcaagtcacgaaagttggtaacacccgaagccggtggcctaaccccttgtgggaggga

SEQ ID NO: 3 - DNA, 1395 bp, Arthrobacter agilis
ttcgacggctccctcccacaaggggttaggccaccggcttcgggtgttaccaactttcgtgacttgacgggcggtgtgtacaaggcccgggaacgtattcaccgcagcgttgctgatctgcgattactagcgactccaacttcatgaggtcgagttgcagacctcaatccgaactgagaccggctttttgggattagctccacctcacagtatcgcaaccctttgtaccggccattgtagcatgcgtgaagcccaagacataaggggcatgatgatttgacgtcgtccccaccttcctccgagttgaccccggcagtctcccatgagtccccggcataacccgctggcaacatggaacgagggttgcgctcgttgcgggacttaacccaacatctcacgacacgagctgacgacaaccatgcaccacctgtaaaccggccacaagtggctgacgcatctctgcgccattccggttcatgtcaagccttggtaaggttcttcgcgttgcatcgaattaatccgcatgctccgccgcttgtgcgggcccccgtcaattcctttgagttttagccttgcggccgtactccccaggcggggcacttaatgcgttagctacggcgcggaaaacgtggaatgtcccccacacctagtgcccaacgtttacggcatggactaccagggtatctaatcctgttcgctccccatgctttcgctcctcagcgtcagttacagcccagagacctgccttcgccatcggtgttcctcctgatatctgcgcatttcaccgctacaccaggaattccagtctcccctactgcactctagtctgcccgtacccaccgcagatccggagttaagccccggactttcacggcagacgcgacaaaccgcctacgagctctttacgcccaataattccggataacgcttgcgccctacgtattaccgcggctgctggcacgtagttagccggcgcttcttctgcaggtaccgtcactttcgcttcttccctactgaaagaggtttacaacccgaaggccttcatccctcacgcggcgtcgctgcatcaggcttgcgcccattgtgcaatattccccactgctgcctcccgtaggagtctgggccgtgtctcagtcccagtgtggccggtcaccctctcaggccggctacccgtcgtcgccttggtgggccattaccccgccaacaagctgataggccgcgagtccatccaaaaccgcaataaagctttccaccaccaggccatgcggccggcagtcatatccggtattagacccggtttcccaggcttatcccagagtcaagggcaggttactcacgtgttactcacccgttcgccactaatccaccagcaagctggcttcatcgttcgactgc